European Patent Specification EP 3 455 368 B1, published November 29, 2023. Title: METHODS AND COMPOSITIONS FOR CLASSIFYING DLBCL. Applicant: Roche Diagnostics GmbH F. Hoffmann-La Roche AG Roche Molecular Systems, Inc. The sequence listing filed with the application follows.

SEQUENCE LISTING (314 sequences)

SEQ ID NO: 1 - DNA, 20 bp, Artificial Sequence
  source: /note="Description of Artificial Sequence: Synthetic primer"
ggcagtattgacagggagga

SEQ ID NO: 2 - DNA, 19 bp, Artificial Sequence
  source: /note="Description of Artificial Sequence: Synthetic primer"
tggtttacccacaggctga

SEQ ID NO: 3 - DNA, 21 bp, Artificial Sequence
  source: /note="Description of Artificial Sequence: Synthetic primer"
ggagaaggccaatttggagat

SEQ ID NO: 4 - DNA, 28 bp, Artificial Sequence
  source: /note="Description of Artificial Sequence: Synthetic primer"
acagtttttacatgttttaattgcaacc

SEQ ID NO: 5 - DNA, 25 bp, Artificial Sequence
  source: /note="Description of Artificial Sequence: Synthetic primer"
ggacagaaaaggaatgctacaacta

SEQ ID NO: 6 - DNA, 20 bp, Artificial Sequence
  source: /note="Description of Artificial Sequence: Synthetic primer"
cgcaatggttagggatggtg

SEQ ID NO: 7 - DNA, 21 bp, Artificial Sequence
  source: /note="Description of Artificial Sequence: Synthetic primer"
agcttagtacagctcttgcat

SEQ ID NO: 8 - DNA, 23 bp, Artificial Sequence
  source: /note="Description of Artificial Sequence: Synthetic primer"
tcatttgaggacaccagaacatt

SEQ ID NO: 9 - DNA, 21 bp, Artificial Sequence
  source: /note="Description of Artificial Sequence: Synthetic primer"
gcccagaagaaggaatcagtt

SEQ ID NO: 10 - DNA, 21 bp, Artificial Sequence
  source: /note="Description of Artificial Sequence: Synthetic primer"
ggtttgcacttgagtgaagtc

SEQ ID NO: 11 - DNA, 19 bp, Artificial Sequence
  source: /note="Description of Artificial Sequence: Synthetic primer"
accattcccctcctaccag

SEQ ID NO: 12 - DNA, 20 bp, Artificial Sequence
  source: /note="Description of Artificial Sequence: Synthetic primer"
ctcacccaggtcagagttca

SEQ ID NO: 13 - DNA, 21 bp, Artificial Sequence
  source: /note="Description of Artificial Sequence: Synthetic primer"
gacctcaggagatagcaatgt

SEQ ID NO: 14 - DNA, 18 bp, Artificial Sequence
  source: /note="Description of Artificial Sequence: Synthetic primer"
cacttgcccaatccctcg

SEQ ID NO: 15 - DNA, 20 bp, Artificial Sequence
  source: /note="Description of Artificial Sequence: Synthetic primer"
gaatggaacctcgcagtcat

SEQ ID NO: 16 - DNA, 21 bp, Artificial Sequence
  source: /note="Description of Artificial Sequence: Synthetic primer"
ggccaactttggtattgatgg

SEQ ID NO: 17 - DNA, 20 bp, Artificial Sequence
  source: /note="Description of Artificial Sequence: Synthetic primer"
ttcgacgttttacctcagct

SEQ ID NO: 18 - DNA, 20 bp, Artificial Sequence
  source: /note="Description of Artificial Sequence: Synthetic primer"
ggcttcacaccatgcatcag

SEQ ID NO: 19 - DNA, 20 bp, Artificial Sequence
  source: /note="Description of Artificial Sequence: Synthetic primer"
gaaagaaggtgaacgggctt

SEQ ID NO: 20 - DNA, 18 bp, Artificial Sequence
  source: /note="Description of Artificial Sequence: Synthetic primer"
gtgtgtccgcatgccttg

SEQ ID NO: 21 - DNA, 22 bp, Artificial Sequence
  source: /note="Description of Artificial Sequence: Synthetic primer"
cctgtctggataatcatggagc

SEQ ID NO: 22 - DNA, 26 bp, Artificial Sequence
  source: /note="Description of Artificial Sequence: Synthetic primer"
gctagatccaaactgtatttccttac

SEQ ID NO: 23 - DNA, 19 bp, Artificial Sequence
  source: /note="Description of Artificial Sequence: Synthetic primer"
cggcccaggtttactgaac

SEQ ID NO: 24 - DNA, 21 bp, Artificial Sequence
  source: /note="Description of Artificial Sequence: Synthetic primer"
tcttcttgctgagccttctct

SEQ ID NO: 25 - DNA, 20 bp, Artificial Sequence
  source: /note="Description of Artificial Sequence: Synthetic primer"
caggctgcatcaggatgaat

SEQ ID NO: 26 - DNA, 18 bp, Artificial Sequence
  source: /note="Description of Artificial Sequence: Synthetic primer"
cagcaggctctcaggaca

SEQ ID NO: 27 - DNA, 19 bp, Artificial Sequence
  source: /note="Description of Artificial Sequence: Synthetic primer"
ctctcaggctgcatcagga

SEQ ID NO: 28 - DNA, 18 bp, Artificial Sequence
  source: /note="Description of Artificial Sequence: Synthetic primer"
cagcaggctctcaggaca

SEQ ID NO: 29 - DNA, 20 bp, Artificial Sequence
  source: /note="Description of Artificial Sequence: Synthetic primer"
acaagatcagcttctcccac

SEQ ID NO: 30 - DNA, 21 bp, Artificial Sequence
  source: /note="Description of Artificial Sequence: Synthetic primer"
ctcgtagagtcttggaatgca

SEQ ID NO: 31 - DNA, 20 bp, Artificial Sequence
  source: /note="Description of Artificial Sequence: Synthetic primer"
caagatcagcttctcccacg

SEQ ID NO: 32 - DNA, 23 bp, Artificial Sequence
  source: /note="Description of Artificial Sequence: Synthetic primer"
ctcgtagagtcttggaatgcaat

SEQ ID NO: 33 - DNA, 25 bp, Artificial Sequence
  source: /note="Description of Artificial Sequence: Synthetic primer"
aggaaccagaaacaatagaagaaca

SEQ ID NO: 34 - DNA, 22 bp, Artificial Sequence
  source: /note="Description of Artificial Sequence: Synthetic primer"
cgatttcacagtggttacagga

SEQ ID NO: 35 - DNA, 21 bp, Artificial Sequence
  source: /note="Description of Artificial Sequence: Synthetic primer"
gccaaagaggaaccagaaaca

SEQ ID NO: 36 - DNA, 21 bp, Artificial Sequence
  source: /note="Description of Artificial Sequence: Synthetic primer"
accgatttcacagtggttaca

SEQ ID NO: 37 - DNA, 20 bp, Artificial Sequence
  source: /note="Description of Artificial Sequence: Synthetic primer"
cagtagggctgagatgttgg

SEQ ID NO: 38 - DNA, 22 bp, Artificial Sequence
  source: /note="Description of Artificial Sequence: Synthetic primer"
acgtgctgaatcatcacttcaa

SEQ ID NO: 39 - DNA, 18 bp, Artificial Sequence
  source: /note="Description of Artificial Sequence: Synthetic primer"
ggccagtagggctgagat

SEQ ID NO: 40 - DNA, 22 bp, Artificial Sequence
  source: /note="Description of Artificial Sequence: Synthetic primer"
acgtgctgaatcatcacttcaa

SEQ ID NO: 41 - DNA, 24 bp, Artificial Sequence
  source: /note="Description of Artificial Sequence: Synthetic primer"
gactgccaaattaaaaaacgttca

SEQ ID NO: 42 - DNA, 24 bp, Artificial Sequence
  source: /note="Description of Artificial Sequence: Synthetic primer"
tttctgggtaaagaggcaatagtc

SEQ ID NO: 43 - DNA, 23 bp, Artificial Sequence
  source: /note="Description of Artificial Sequence: Synthetic primer"
ggaagccaagtctttctgaaaag

SEQ ID NO: 44 - DNA, 21 bp, Artificial Sequence
  source: /note="Description of Artificial Sequence: Synthetic primer"
gaggacttgagatttgttgcc

SEQ ID NO: 45 - DNA, 26 bp, Artificial Sequence
  source: /note="Description of Artificial Sequence: Synthetic primer"
ggcagaagaaaatttgaagaaagaaa

SEQ ID NO: 46 - DNA, 20 bp, Artificial Sequence
  source: /note="Description of Artificial Sequence: Synthetic primer"
aatgatttcctgtgcctggt

SEQ ID NO: 47 - DNA, 21 bp, Artificial Sequence
  source: /note="Description of Artificial Sequence: Synthetic primer"
ggtggctgggatggaaaataa

SEQ ID NO: 48 - DNA, 19 bp, Artificial Sequence
  source: /note="Description of Artificial Sequence: Synthetic primer"
ggacggtgttcactctgct

SEQ ID NO: 49 - DNA, 19 bp, Artificial Sequence
  source: /note="Description of Artificial Sequence: Synthetic primer"
gaagagccacctgcgaatc

SEQ ID NO: 50 - DNA, 20 bp, Artificial Sequence
  source: /note="Description of Artificial Sequence: Synthetic primer"
gctggcttttgtgacggaaa

SEQ ID NO: 51 - DNA, 18 bp, Artificial Sequence
  source: /note="Description of Artificial Sequence: Synthetic primer"
ccacctgcgaatccacac

SEQ ID NO: 52 - DNA, 21 bp, Artificial Sequence
  source: /note="Description of Artificial Sequence: Synthetic primer"
ctggcttttgtgacggaaatg

SEQ ID NO: 53 - DNA, 19 bp, Artificial Sequence
  source: /note="Description of Artificial Sequence: Synthetic primer"
gaagagccacctgcgaatc

SEQ ID NO: 54 - DNA, 19 bp, Artificial Sequence
  source: /note="Description of Artificial Sequence: Synthetic primer"
gctggcttttgtgacggaa

SEQ ID NO: 55 - DNA, 18 bp, Artificial Sequence
  source: /note="Description of Artificial Sequence: Synthetic primer"
ccacctgcgaatccacac

SEQ ID NO: 56 - DNA, 20 bp, Artificial Sequence
  source: /note="Description of Artificial Sequence: Synthetic primer"
gctggcttttgtgacggaaa

SEQ ID NO: 57 - DNA, 19 bp, Artificial Sequence
  source: /note="Description of Artificial Sequence: Synthetic primer"
catgttgtggacacttgcc

SEQ ID NO: 58 - DNA, 20 bp, Artificial Sequence
  source: /note="Description of Artificial Sequence: Synthetic primer"
cttcacgaggaggcttgatg

SEQ ID NO: 59 - DNA, 20 bp, Artificial Sequence
  source: /note="Description of Artificial Sequence: Synthetic primer"
ggagcatgttgtggacactt

SEQ ID NO: 60 - DNA, 20 bp, Artificial Sequence
  source: /note="Description of Artificial Sequence: Synthetic primer"
ctcttcacgaggaggcttga

SEQ ID NO: 61 - DNA, 20 bp, Artificial Sequence
  source: /note="Description of Artificial Sequence: Synthetic primer"
atggagcatgttgtggacac

SEQ ID NO: 62 - DNA, 18 bp, Artificial Sequence
  source: /note="Description of Artificial Sequence: Synthetic primer"
cgaggaggcttgatggca

SEQ ID NO: 63 - DNA, 19 bp, Artificial Sequence
  source: /note="Description of Artificial Sequence: Synthetic primer"
ggactccaccatcccacaa

SEQ ID NO: 64 - DNA, 20 bp, Artificial Sequence
  source: /note="Description of Artificial Sequence: Synthetic primer"
tagagtggtgagtggctctc

SEQ ID NO: 65 - DNA, 18 bp, Artificial Sequence
  source: /note="Description of Artificial Sequence: Synthetic primer"
gtgccctgcttcatgatg

SEQ ID NO: 66 - DNA, 21 bp, Artificial Sequence
  source: /note="Description of Artificial Sequence: Synthetic primer"
ctggtgtcgagagatccactc

SEQ ID NO: 67 - DNA, 18 bp, Artificial Sequence
  source: /note="Description of Artificial Sequence: Synthetic primer"
ggctgtgccaaactcatt

SEQ ID NO: 68 - DNA, 17 bp, Artificial Sequence
  source: /note="Description of Artificial Sequence: Synthetic primer"
gggctgtacacccttgt

SEQ ID NO: 69 - DNA, 18 bp, Artificial Sequence
  source: /note="Description of Artificial Sequence: Synthetic primer"
gtgccctgcttcatgatg

SEQ ID NO: 70 - DNA, 21 bp, Artificial Sequence
  source: /note="Description of Artificial Sequence: Synthetic primer"
catggtactggtgtcgagaga

SEQ ID NO: 71 - DNA, 18 bp, Artificial Sequence
  source: /note="Description of Artificial Sequence: Synthetic primer"
gtgccctgcttcatgatg

SEQ ID NO: 72 - DNA, 18 bp, Artificial Sequence
  source: /note="Description of Artificial Sequence: Synthetic primer"
ccgggagtgcatggtact

SEQ ID NO: 73 - DNA, 18 bp, Artificial Sequence
  source: /note="Description of Artificial Sequence: Synthetic primer"
ggacaccgcctcacagat

SEQ ID NO: 74 - DNA, 20 bp, Artificial Sequence
  source: /note="Description of Artificial Sequence: Synthetic primer"
agtgggcatgtgactgagtc

SEQ ID NO: 75 - DNA, 18 bp, Artificial Sequence
  source: /note="Description of Artificial Sequence: Synthetic primer"
ggacaccgcctcacagat

SEQ ID NO: 76 - DNA, 18 bp, Artificial Sequence
  source: /note="Description of Artificial Sequence: Synthetic primer"
cttcgagtgggcatgtga

SEQ ID NO: 77 - DNA, 18 bp, Artificial Sequence
  source: /note="Description of Artificial Sequence: Synthetic primer"
cgcctcacagatcgactc

SEQ ID NO: 78 - DNA, 18 bp, Artificial Sequence
  source: /note="Description of Artificial Sequence: Synthetic primer"
gcagtgcgacttcgagtg

SEQ ID NO: 79 - DNA, 18 bp, Artificial Sequence
  source: /note="Description of Artificial Sequence: Synthetic primer"
accgtcttcgcaggacac

SEQ ID NO: 80 - DNA, 19 bp, Artificial Sequence
  source: /note="Description of Artificial Sequence: Synthetic primer"
gggcatgtgactgagtctg

SEQ ID NO: 81 - DNA, 19 bp, Artificial Sequence
  source: /note="Description of Artificial Sequence: Synthetic primer"
ggcgactggacttacgagg

SEQ ID NO: 82 - DNA, 21 bp, Artificial Sequence
  source: /note="Description of Artificial Sequence: Synthetic primer"
ccaggaattccttcctcttgg

SEQ ID NO: 83 - DNA, 20 bp, Artificial Sequence
  source: /note="Description of Artificial Sequence: Synthetic primer"
tcctggatgacttgttcagc

SEQ ID NO: 84 - DNA, 20 bp, Artificial Sequence
  source: /note="Description of Artificial Sequence: Synthetic primer"
aggacctgtttggccatgat

SEQ ID NO: 85 - DNA, 18 bp, Artificial Sequence
  source: /note="Description of Artificial Sequence: Synthetic primer"
acgtccatcaccagtgca

SEQ ID NO: 86 - DNA, 20 bp, Artificial Sequence
  source: /note="Description of Artificial Sequence: Synthetic primer"
cttctcacactcgtaggggt

SEQ ID NO: 87 - DNA, 18 bp, Artificial Sequence
  source: /note="Description of Artificial Sequence: Synthetic primer"
acgtccatcaccagtgca

SEQ ID NO: 88 - DNA, 19 bp, Artificial Sequence
  source: /note="Description of Artificial Sequence: Synthetic primer"
cccgcttctcacactcgta

SEQ ID NO: 89 - DNA, 19 bp, Artificial Sequence
  source: /note="Description of Artificial Sequence: Synthetic primer"
cagctgcccatgagcattc

SEQ ID NO: 90 - DNA, 20 bp, Artificial Sequence
  source: /note="Description of Artificial Sequence: Synthetic primer"
tcaggttcacagcagagtcc

SEQ ID NO: 91 - DNA, 19 bp, Artificial Sequence
  source: /note="Description of Artificial Sequence: Synthetic primer"
cagctgcccatgagcattc

SEQ ID NO: 92 - DNA, 19 bp, Artificial Sequence
  source: /note="Description of Artificial Sequence: Synthetic primer"
cgtcaggttcacagcagag

SEQ ID NO: 93 - DNA, 20 bp, Artificial Sequence
  source: /note="Description of Artificial Sequence: Synthetic primer"
agcatgtcggtggagatcaa

SEQ ID NO: 94 - DNA, 18 bp, Artificial Sequence
  source: /note="Description of Artificial Sequence: Synthetic primer"
ttgggagcagaggttggc

SEQ ID NO: 95 - DNA, 20 bp, Artificial Sequence
  source: /note="Description of Artificial Sequence: Synthetic primer"
atcagcatgtcggtggagat

SEQ ID NO: 96 - DNA, 20 bp, Artificial Sequence
  source: /note="Description of Artificial Sequence: Synthetic primer"
tttgttgggagcagaggttg

SEQ ID NO: 97 - DNA, 21 bp, Artificial Sequence
  source: /note="Description of Artificial Sequence: Synthetic primer"
aggacatccaaccctacatgc

SEQ ID NO: 98 - DNA, 20 bp, Artificial Sequence
  source: /note="Description of Artificial Sequence: Synthetic primer"
gaagacctcttcttcgcact

SEQ ID NO: 99 - DNA, 20 bp, Artificial Sequence
  source: /note="Description of Artificial Sequence: Synthetic primer"
cttcattgctctgtgtgcca

SEQ ID NO: 100 - DNA, 19 bp, Artificial Sequence
  source: /note="Description of Artificial Sequence: Synthetic primer"
tgctcccacacttccagtt

SEQ ID NO: 101 - DNA, 20 bp, Artificial Sequence
  source: /note="Description of Artificial Sequence: Synthetic primer"
cttcattgctctgtgtgcca

SEQ ID NO: 102 - DNA, 20 bp, Artificial Sequence
  source: /note="Description of Artificial Sequence: Synthetic primer"
ccacacttccagttgcgatc

SEQ ID NO: 103 - DNA, 20 bp, Artificial Sequence
  source: /note="Description of Artificial Sequence: Synthetic primer"
gactgagctgctggctaaga

SEQ ID NO: 104 - DNA, 18 bp, Artificial Sequence
  source: /note="Description of Artificial Sequence: Synthetic primer"
gagcaccgcctcaatctg

SEQ ID NO: 105 - DNA, 20 bp, Artificial Sequence
  source: /note="Description of Artificial Sequence: Synthetic primer"
ggacatccaaccctacatgc

SEQ ID NO: 106 - DNA, 21 bp, Artificial Sequence
  source: /note="Description of Artificial Sequence: Synthetic primer"
agagggaagacctcttcttcg

SEQ ID NO: 107 - DNA, 20 bp, Artificial Sequence
  source: /note="Description of Artificial Sequence: Synthetic primer"
ggacatccaaccctacatgc

SEQ ID NO: 108 - DNA, 21 bp, Artificial Sequence
  source: /note="Description of Artificial Sequence: Synthetic primer"
ggaagacctcttcttcgcact

SEQ ID NO: 109 - DNA, 20 bp, Artificial Sequence
  source: /note="Description of Artificial Sequence: Synthetic primer"
cttcattgctctgtgtgcca

SEQ ID NO: 110 - DNA, 19 bp, Artificial Sequence
  source: /note="Description of Artificial Sequence: Synthetic primer"
ctgctcccacacttccagt

SEQ ID NO: 111 - DNA, 20 bp, Artificial Sequence
  source: /note="Description of Artificial Sequence: Synthetic primer"
accttcattgctctgtgtgc

SEQ ID NO: 112 - DNA, 19 bp, Artificial Sequence
  source: /note="Description of Artificial Sequence: Synthetic primer"
gctcccacacttccagttg

SEQ ID NO: 113 - DNA, 18 bp, Artificial Sequence
  source: /note="Description of Artificial Sequence: Synthetic primer"
aaggacctgcctctgtcg

SEQ ID NO: 114 - DNA, 20 bp, Artificial Sequence
  source: /note="Description of Artificial Sequence: Synthetic primer"
tctcctctgccatcttcagg

SEQ ID NO: 115 - DNA, 18 bp, Artificial Sequence
  source: /note="Description of Artificial Sequence: Synthetic primer"
ccaaggacctgcctctgt

SEQ ID NO: 116 - DNA, 20 bp, Artificial Sequence
  source: /note="Description of Artificial Sequence: Synthetic primer"
ctcctctgccatcttcaggg

SEQ ID NO: 117 - DNA, 19 bp, Artificial Sequence
  source: /note="Description of Artificial Sequence: Synthetic primer"
ccaaggacctgcctctgtc

SEQ ID NO: 118 - DNA, 20 bp, Artificial Sequence
  source: /note="Description of Artificial Sequence: Synthetic primer"
tctcctctgccatcttcagg

SEQ ID NO: 119 - DNA, 19 bp, Artificial Sequence
  source: /note="Description of Artificial Sequence: Synthetic primer"
ccaaggacctgcctctgtc

SEQ ID NO: 120 - DNA, 20 bp, Artificial Sequence
  source: /note="Description of Artificial Sequence: Synthetic primer"
ctcctctgccatcttcaggg

SEQ ID NO: 121 - DNA, 19 bp, Artificial Sequence
  source: /note="Description of Artificial Sequence: Synthetic primer"
caaggacctgcctctgtcg

SEQ ID NO: 122 - DNA, 20 bp, Artificial Sequence
  source: /note="Description of Artificial Sequence: Synthetic primer"
tctcctctgccatcttcagg

SEQ ID NO: 123 - DNA, 18 bp, Artificial Sequence
  source: /note="Description of Artificial Sequence: Synthetic primer"
ccaaggacctgcctctgt

SEQ ID NO: 124 - DNA, 20 bp, Artificial Sequence
  source: /note="Description of Artificial Sequence: Synthetic primer"
ctctgccatcttcaggggat

SEQ ID NO: 125 - DNA, 18 bp, Artificial Sequence
  source: /note="Description of Artificial Sequence: Synthetic primer"
aaggacctgcctctgtcg

SEQ ID NO: 126 - DNA, 20 bp, Artificial Sequence
  source: /note="Description of Artificial Sequence: Synthetic primer"
tgctctcctctgccatcttc

SEQ ID NO: 127 - DNA, 19 bp, Artificial Sequence
  source: /note="Description of Artificial Sequence: Synthetic primer"
ccaaggacctgcctctgtc

SEQ ID NO: 128 - DNA, 20 bp, Artificial Sequence
  source: /note="Description of Artificial Sequence: Synthetic primer"
ctctgccatcttcaggggat

SEQ ID NO: 129 - DNA, 20 bp, Artificial Sequence
  source: /note="Description of Artificial Sequence: Synthetic primer"
aaaccagcaaccagcacttt

SEQ ID NO: 130 - DNA, 19 bp, Artificial Sequence
  source: /note="Description of Artificial Sequence: Synthetic primer"
gaggagctccaagggtcac

SEQ ID NO: 131 - DNA, 20 bp, Artificial Sequence
  source: /note="Description of Artificial Sequence: Synthetic primer"
caaccagcactttccctagc

SEQ ID NO: 132 - DNA, 19 bp, Artificial Sequence
  source: /note="Description of Artificial Sequence: Synthetic primer"
ccactggaggagctccaag

SEQ ID NO: 133 - DNA, 19 bp, Artificial Sequence
  source: /note="Description of Artificial Sequence: Synthetic primer"
acttcccctgacctgaacc

SEQ ID NO: 134 - DNA, 20 bp, Artificial Sequence
  source: /note="Description of Artificial Sequence: Synthetic primer"
gagacactctgcccctgtag

SEQ ID NO: 135 - DNA, 19 bp, Artificial Sequence
  source: /note="Description of Artificial Sequence: Synthetic primer"
cgacttcccctgacctgaa

SEQ ID NO: 136 - DNA, 20 bp, Artificial Sequence
  source: /note="Description of Artificial Sequence: Synthetic primer"
gagacactctgcccctgtag

SEQ ID NO: 137 - DNA, 20 bp, Artificial Sequence
  source: /note="Description of Artificial Sequence: Synthetic primer"
gcaaccagcactttccctag

SEQ ID NO: 138 - DNA, 20 bp, Artificial Sequence
  source: /note="Description of Artificial Sequence: Synthetic primer"
attcatcccactggaggagc

SEQ ID NO: 139 - DNA, 18 bp, Artificial Sequence
  source: /note="Description of Artificial Sequence: Synthetic primer"
tggccgtcatcctcagtc

SEQ ID NO: 140 - DNA, 21 bp, Artificial Sequence
  source: /note="Description of Artificial Sequence: Synthetic primer"
cctcccttcttttcagacacg

SEQ ID NO: 141 - DNA, 19 bp, Artificial Sequence
  source: /note="Description of Artificial Sequence: Synthetic primer"
gtggccgtcatcctcagtc

SEQ ID NO: 142 - DNA, 20 bp, Artificial Sequence
  source: /note="Description of Artificial Sequence: Synthetic primer"
tcttttcagacacgcagctt

SEQ ID NO: 143 - DNA, 18 bp, Artificial Sequence
  source: /note="Description of Artificial Sequence: Synthetic primer"
gtggccgtcatcctcagt

SEQ ID NO: 144 - DNA, 20 bp, Artificial Sequence
  source: /note="Description of Artificial Sequence: Synthetic primer"
tcttttcagacacgcagctt

SEQ ID NO: 145 - DNA, 26 bp, Artificial Sequence
  source: /note="Description of Artificial Sequence: Synthetic primer"
tcaagtcaaaaattccaaatgaacac

SEQ ID NO: 146 - DNA, 20 bp, Artificial Sequence
  source: /note="Description of Artificial Sequence: Synthetic primer"
tggaagtttcatggcactga

SEQ ID NO: 147 - DNA, 19 bp, Artificial Sequence
  source: /note="Description of Artificial Sequence: Synthetic primer"
taccagccagtccagacac

SEQ ID NO: 148 - DNA, 21 bp, Artificial Sequence
  source: /note="Description of Artificial Sequence: Synthetic primer"
tcggataaacagaacgtcctt

SEQ ID NO: 149 - DNA, 22 bp, Artificial Sequence
  source: /note="Description of Artificial Sequence: Synthetic primer"
ggcttcaggaactcaatgaaga

SEQ ID NO: 150 - DNA, 23 bp, Artificial Sequence
  source: /note="Description of Artificial Sequence: Synthetic primer"
caggacttctactgtcttttcca

SEQ ID NO: 151 - DNA, 22 bp, Artificial Sequence
  source: /note="Description of Artificial Sequence: Synthetic primer"
ggcttcaggaactcaatgaaga

SEQ ID NO: 152 - DNA, 20 bp, Artificial Sequence
  source: /note="Description of Artificial Sequence: Synthetic primer"
ggcgttccaggacttctact

SEQ ID NO: 153 - DNA, 23 bp, Artificial Sequence
  source: /note="Description of Artificial Sequence: Synthetic primer"
gggaatgatatggtgttctgtga

SEQ ID NO: 154 - DNA, 19 bp, Artificial Sequence
  source: /note="Description of Artificial Sequence: Synthetic primer"
ccttctgggaccttgagga

SEQ ID NO: 155 - DNA, 21 bp, Artificial Sequence
  source: /note="Description of Artificial Sequence: Synthetic primer"
actaaatgggctcatgtcagc

SEQ ID NO: 156 - DNA, 20 bp, Artificial Sequence
  source: /note="Description of Artificial Sequence: Synthetic primer"
atcggttccatcctctcagg

SEQ ID NO: 157 - DNA, 23 bp, Artificial Sequence
  source: /note="Description of Artificial Sequence: Synthetic primer"
tgagaatgtttatgcatctacgc

SEQ ID NO: 158 - DNA, 22 bp, Artificial Sequence
  source: /note="Description of Artificial Sequence: Synthetic primer"
agcttctctcgtctgcttatca

SEQ ID NO: 159 - DNA, 20 bp, Artificial Sequence
  source: /note="Description of Artificial Sequence: Synthetic primer"
ggtttgcaagtccagcttct

SEQ ID NO: 160 - DNA, 22 bp, Artificial Sequence
  source: /note="Description of Artificial Sequence: Synthetic primer"
tggtgggtaaaacagtgagttt

SEQ ID NO: 161 - DNA, 18 bp, Artificial Sequence
  source: /note="Description of Artificial Sequence: Synthetic primer"
gccaccaggaacacccat

SEQ ID NO: 162 - DNA, 20 bp, Artificial Sequence
  source: /note="Description of Artificial Sequence: Synthetic primer"
ggtccaggaggtactgcatt

SEQ ID NO: 163 - DNA, 28 bp, Artificial Sequence
  source: /note="Description of Artificial Sequence: Synthetic primer"
acatgtatactttaatgaatgcagtacc

SEQ ID NO: 164 - DNA, 18 bp, Artificial Sequence
  source: /note="Description of Artificial Sequence: Synthetic primer"
tgggaccatctgacccag

SEQ ID NO: 165 - DNA, 29 bp, Artificial Sequence
  source: /note="Description of Artificial Sequence: Synthetic primer"
aacatgtatactttaatgaatgcagtacc

SEQ ID NO: 166 - DNA, 19 bp, Artificial Sequence
  source: /note="Description of Artificial Sequence: Synthetic primer"
atgggaccatctgacccag

SEQ ID NO: 167 - DNA, 18 bp, Artificial Sequence
  source: /note="Description of Artificial Sequence: Synthetic primer"
gccaccaggaacacccat

SEQ ID NO: 168 - DNA, 21 bp, Artificial Sequence
  source: /note="Description of Artificial Sequence: Synthetic primer"
ccaggaggtactgcattcatt

SEQ ID NO: 169 - DNA, 18 bp, Artificial Sequence
  source: /note="Description of Artificial Sequence: Synthetic primer"
gccaccaggaacacccat

SEQ ID NO: 170 - DNA, 21 bp, Artificial Sequence
  source: /note="Description of Artificial Sequence: Synthetic primer"
gtccaggaggtactgcattca

SEQ ID NO: 171 - DNA, 28 bp, Artificial Sequence
  source: /note="Description of Artificial Sequence: Synthetic primer"
acatgtatactttaatgaatgcagtacc

SEQ ID NO: 172 - DNA, 19 bp, Artificial Sequence
  source: /note="Description of Artificial Sequence: Synthetic primer"
atgggaccatctgacccag

SEQ ID NO: 173 - DNA, 18 bp, Artificial Sequence
  source: /note="Description of Artificial Sequence: Synthetic primer"
gccaccaggaacacccat

SEQ ID NO: 174 - DNA, 22 bp, Artificial Sequence
  source: /note="Description of Artificial Sequence: Synthetic primer"
tccaggaggtactgcattcatt

SEQ ID NO: 175 - DNA, 18 bp, Artificial Sequence
  source: /note="Description of Artificial Sequence: Synthetic primer"
gccaccaggaacacccat

SEQ ID NO: 176 - DNA, 20 bp, Artificial Sequence
  source: /note="Description of Artificial Sequence: Synthetic primer"
taggtccaggaggtactgca

SEQ ID NO: 177 - DNA, 22 bp, Artificial Sequence
  source: /note="Description of Artificial Sequence: Synthetic primer"
aacagtattacctggtagctcc

SEQ ID NO: 178 - DNA, 20 bp, Artificial Sequence
  source: /note="Description of Artificial Sequence: Synthetic primer"
agggcacataaaccacctga

SEQ ID NO: 179 - DNA, 20 bp, Artificial Sequence
  source: /note="Description of Artificial Sequence: Synthetic primer"
atcgatcccacctgtaacgt

SEQ ID NO: 180 - DNA, 23 bp, Artificial Sequence
  source: /note="Description of Artificial Sequence: Synthetic primer"
caggtaatactgttcacacagca

SEQ ID NO: 181 - DNA, 23 bp, Artificial Sequence
  source: /note="Description of Artificial Sequence: Synthetic primer"
gaacagtattacctggtagctcc

SEQ ID NO: 182 - DNA, 20 bp, Artificial Sequence
  source: /note="Description of Artificial Sequence: Synthetic primer"
gagggcacataaaccacctg

SEQ ID NO: 183 - DNA, 20 bp, Artificial Sequence
  source: /note="Description of Artificial Sequence: Synthetic primer"
atcgatcccacctgtaacgt

SEQ ID NO: 184 - DNA, 23 bp, Artificial Sequence
  source: /note="Description of Artificial Sequence: Synthetic primer"
ccaggtaatactgttcacacagc

SEQ ID NO: 185 - DNA, 23 bp, Artificial Sequence
  source: /note="Description of Artificial Sequence: Synthetic primer"
gaacagtattacctggtagctcc

SEQ ID NO: 186 - DNA, 20 bp, Artificial Sequence
  source: /note="Description of Artificial Sequence: Synthetic primer"
gggcacataaaccacctgaa

SEQ ID NO: 187 - DNA, 22 bp, Artificial Sequence
  source: /note="Description of Artificial Sequence: Synthetic primer"
aacagtattacctggtagctcc

SEQ ID NO: 188 - DNA, 20 bp, Artificial Sequence
  source: /note="Description of Artificial Sequence: Synthetic primer"
gtgagggcacataaaccacc

SEQ ID NO: 189 - DNA, 20 bp, Artificial Sequence
  source: /note="Description of Artificial Sequence: Synthetic primer"
atcgatcccacctgtaacgt

SEQ ID NO: 190 - DNA, 22 bp, Artificial Sequence
  source: /note="Description of Artificial Sequence: Synthetic primer"
caggtaatactgttcacacagc

SEQ ID NO: 191 - DNA, 18 bp, Artificial Sequence
  source: /note="Description of Artificial Sequence: Synthetic primer"
tcgccgctctccatcaaa

SEQ ID NO: 192 - DNA, 21 bp, Artificial Sequence
  source: /note="Description of Artificial Sequence: Synthetic primer"
gcacaggaagttcctttcgta

SEQ ID NO: 193 - DNA, 24 bp, Artificial Sequence
  source: /note="Description of Artificial Sequence: Synthetic primer"
gaagatctctgatgagaagaaccg

SEQ ID NO: 194 - DNA, 22 bp, Artificial Sequence
  source: /note="Description of Artificial Sequence: Synthetic primer"
gcttcccggtcattctttagtt

SEQ ID NO: 195 - DNA, 19 bp, Artificial Sequence
  source: /note="Description of Artificial Sequence: Synthetic primer"
tgccataaagcgcactgac

SEQ ID NO: 196 - DNA, 23 bp, Artificial Sequence
  source: /note="Description of Artificial Sequence: Synthetic primer"
ggcaataaaatccactgatggga

SEQ ID NO: 197 - DNA, 25 bp, Artificial Sequence
  source: /note="Description of Artificial Sequence: Synthetic primer"
gtactatcttaggaccgagttagag

SEQ ID NO: 198 - DNA, 20 bp, Artificial Sequence
  source: /note="Description of Artificial Sequence: Synthetic primer"
gccatccttctcccttcgtt

SEQ ID NO: 199 - DNA, 20 bp, Artificial Sequence
  source: /note="Description of Artificial Sequence: Synthetic primer"
atgccataaagcgcactgac

SEQ ID NO: 200 - DNA, 22 bp, Artificial Sequence
  source: /note="Description of Artificial Sequence: Synthetic primer"
ggcaataaaatccactgatggg

SEQ ID NO: 201 - DNA, 26 bp, Artificial Sequence
  source: /note="Description of Artificial Sequence: Synthetic primer"
tgtactatcttaggaccgagttagag

SEQ ID NO: 202 - DNA, 20 bp, Artificial Sequence
  source: /note="Description of Artificial Sequence: Synthetic primer"
gccatccttctcccttcgtt

SEQ ID NO: 203 - DNA, 24 bp, Artificial Sequence
  source: /note="Description of Artificial Sequence: Synthetic primer"
agatgtactatcttaggaccgagt

SEQ ID NO: 204 - DNA, 20 bp, Artificial Sequence
  source: /note="Description of Artificial Sequence: Synthetic primer"
ccatccttctcccttcgttt

SEQ ID NO: 205 - DNA, 20 bp, Artificial Sequence
  source: /note="Description of Artificial Sequence: Synthetic primer"
gccataaagcgcactgacaa

SEQ ID NO: 206 - DNA, 22 bp, Artificial Sequence
  source: /note="Description of Artificial Sequence: Synthetic primer"
ggcaataaaatccactgatggg

SEQ ID NO: 207 - DNA, 25 bp, Artificial Sequence
  source: /note="Description of Artificial Sequence: Synthetic primer"
gtactatcttaggaccgagttagag

SEQ ID NO: 208 - DNA, 21 bp, Artificial Sequence
  source: /note="Description of Artificial Sequence: Synthetic primer"
ccatccttctcccttcgtttc

SEQ ID NO: 209 - DNA, 21 bp, Artificial Sequence
  source: /note="Description of Artificial Sequence: Synthetic primer"
aagacttacctgcggaaaacg

SEQ ID NO: 210 - DNA, 20 bp, Artificial Sequence
  source: /note="Description of Artificial Sequence: Synthetic primer"
tggcttctttctctcctgct

SEQ ID NO: 211 - DNA, 20 bp, Artificial Sequence
  source: /note="Description of Artificial Sequence: Synthetic primer"
agacttacctgcggaaaacg

SEQ ID NO: 212 - DNA, 20 bp, Artificial Sequence
  source: /note="Description of Artificial Sequence: Synthetic primer"
ttggcttctttctctcctgc

SEQ ID NO: 213 - DNA, 21 bp, Artificial Sequence
  source: /note="Description of Artificial Sequence: Synthetic primer"
aagacttacctgcggaaaacg

SEQ ID NO: 214 - DNA, 21 bp, Artificial Sequence
  source: /note="Description of Artificial Sequence: Synthetic primer"
cttggcttctttctctcctgc

SEQ ID NO: 215 - DNA, 20 bp, Artificial Sequence
  source: /note="Description of Artificial Sequence: Synthetic primer"
gacttacctgcggaaaacgg

SEQ ID NO: 216 - DNA, 20 bp, Artificial Sequence
  source: /note="Description of Artificial Sequence: Synthetic primer"
ttggcttctttctctcctgc

SEQ ID NO: 217 - DNA, 20 bp, Artificial Sequence
  source: /note="Description of Artificial Sequence: Synthetic primer"
agacttacctgcggaaaacg

SEQ ID NO: 218 - DNA, 20 bp, Artificial Sequence
  source: /note="Description of Artificial Sequence: Synthetic primer"
tggcttctttctctcctgct

SEQ ID NO: 219 - DNA, 21 bp, Artificial Sequence
  source: /note="Description of Artificial Sequence: Synthetic primer"
aagacttacctgcggaaaacg

SEQ ID NO: 220 - DNA, 20 bp, Artificial Sequence
  source: /note="Description of Artificial Sequence: Synthetic primer"
ttggcttctttctctcctgc

SEQ ID NO: 221 - DNA, 20 bp, Artificial Sequence
  source: /note="Description of Artificial Sequence: Synthetic primer"
caacgagagtgacagcagtc

SEQ ID NO: 222 - DNA, 21 bp, Artificial Sequence
  source: /note="Description of Artificial Sequence: Synthetic primer"
ggctcttctttgacgtgtaca

SEQ ID NO: 223 - DNA, 20 bp, Artificial Sequence
  source: /note="Description of Artificial Sequence: Synthetic primer"
caacgagagtgacagcagtc

SEQ ID NO: 224 - DNA, 20 bp, Artificial Sequence
  source: /note="Description of Artificial Sequence: Synthetic primer"
gggctcttctttgacgtgta

SEQ ID NO: 225 - DNA, 19 bp, Artificial Sequence
  source: /note="Description of Artificial Sequence: Synthetic primer"
cgcctactgcacacctctc

SEQ ID NO: 226 - DNA, 23 bp, Artificial Sequence
  source: /note="Description of Artificial Sequence: Synthetic primer"
catggaagcggtagtgtatagag

SEQ ID NO: 227 - DNA, 19 bp, Artificial Sequence
  source: /note="Description of Artificial Sequence: Synthetic primer"
cgcctactgcacacctctc

SEQ ID NO: 228 - DNA, 22 bp, Artificial Sequence
  source: /note="Description of Artificial Sequence: Synthetic primer"
ccatggaagcggtagtgtatag

SEQ ID NO: 229 - DNA, 19 bp, Artificial Sequence
  source: /note="Description of Artificial Sequence: Synthetic primer"
cgcctactgcacacctctc

SEQ ID NO: 230 - DNA, 19 bp, Artificial Sequence
  source: /note="Description of Artificial Sequence: Synthetic primer"
ccatggaagcggtagtgta

SEQ ID NO: 231 - DNA, 18 bp, Artificial Sequence
  source: /note="Description of Artificial Sequence: Synthetic primer"
agagcagccacgcctact

SEQ ID NO: 232 - DNA, 23 bp, Artificial Sequence
  source: /note="Description of Artificial Sequence: Synthetic primer"
catggaagcggtagtgtatagag

SEQ ID NO: 233 - DNA, 19 bp, Artificial Sequence
  source: /note="Description of Artificial Sequence: Synthetic primer"
cgaaggccacaaaagatca

SEQ ID NO: 234 - DNA, 20 bp, Artificial Sequence
  source: /note="Description of Artificial Sequence: Synthetic primer"
gcattgagaggtgtgcagta

SEQ ID NO: 235 - DNA, 25 bp, Artificial Sequence
  source: /note="Description of Artificial Sequence: Synthetic primer"
atggacagtggatgaagtagaattc

SEQ ID NO: 236 - DNA, 23 bp, Artificial Sequence
  source: /note="Description of Artificial Sequence: Synthetic primer"
gctgctctgcatgtttttaataa

SEQ ID NO: 237 - DNA, 20 bp, Artificial Sequence
  source: /note="Description of Artificial Sequence: Synthetic primer"
tcttcccatttcagacagca

SEQ ID NO: 238 - DNA, 20 bp, Artificial Sequence
  source: /note="Description of Artificial Sequence: Synthetic primer"
gaggactggaagcactgttt

SEQ ID NO: 239 - DNA, 20 bp, Artificial Sequence
  source: /note="Description of Artificial Sequence: Synthetic primer"
tcttcccatttcagacagca

SEQ ID NO: 240 - DNA, 19 bp, Artificial Sequence
  source: /note="Description of Artificial Sequence: Synthetic primer"
ggaggactggaagcactgt

SEQ ID NO: 241 - DNA, 21 bp, Artificial Sequence
  source: /note="Description of Artificial Sequence: Synthetic primer"
agcaagagtctgggtcttcta

SEQ ID NO: 242 - DNA, 20 bp, Artificial Sequence
  source: /note="Description of Artificial Sequence: Synthetic primer"
gtttcagtcactgggctgac

SEQ ID NO: 243 - DNA, 20 bp, Artificial Sequence
  source: /note="Description of Artificial Sequence: Synthetic primer"
agcaagagtctgggtcttct

SEQ ID NO: 244 - DNA, 19 bp, Artificial Sequence
  source: /note="Description of Artificial Sequence: Synthetic primer"
tttcagtcactgggctgac

SEQ ID NO: 245 - DNA, 21 bp, Artificial Sequence
  source: /note="Description of Artificial Sequence: Synthetic primer"
acagaaacctgtagctgttcc

SEQ ID NO: 246 - DNA, 23 bp, Artificial Sequence
  source: /note="Description of Artificial Sequence: Synthetic primer"
gctctttggctaatagttctgca

SEQ ID NO: 247 - DNA, 21 bp, Artificial Sequence
  source: /note="Description of Artificial Sequence: Synthetic primer"
acagaaacctgtagctgttcc

SEQ ID NO: 248 - DNA, 22 bp, Artificial Sequence
  source: /note="Description of Artificial Sequence: Synthetic primer"
gctctttggctaatagttctgc

SEQ ID NO: 249 - DNA, 20 bp, Artificial Sequence
  source: /note="Description of Artificial Sequence: Synthetic primer"
aattctcagctggcaggttc

SEQ ID NO: 250 - DNA, 23 bp, Artificial Sequence
  source: /note="Description of Artificial Sequence: Synthetic primer"
gattcaaagtcttttcggacaca

SEQ ID NO: 251 - DNA, 20 bp, Artificial Sequence
  source: /note="Description of Artificial Sequence: Synthetic primer"
tgggctcctcctagatttca

SEQ ID NO: 252 - DNA, 21 bp, Artificial Sequence
  source: /note="Description of Artificial Sequence: Synthetic primer"
agaaaaaattctgggctgcca

SEQ ID NO: 253 - DNA, 27 bp, Artificial Sequence
  source: /note="Description of Artificial Sequence: Synthetic probe"
caagggctgcaatcccacacatcttgc

SEQ ID NO: 254 - DNA, 30 bp, Artificial Sequence
  source: /note="Description of Artificial Sequence: Synthetic probe"
aagtcttcagggtccgattggaaaccaaca

SEQ ID NO: 255 - DNA, 35 bp, Artificial Sequence
  source: /note="Description of Artificial Sequence: Synthetic probe"
aggcatttatatgagtccagagaatccagctttgg

SEQ ID NO: 256 - DNA, 23 bp, Artificial Sequence
  source: /note="Description of Artificial Sequence: Synthetic probe"
aggtgcacccgagcctctgacag

SEQ ID NO: 257 - DNA, 33 bp, Artificial Sequence
  source: /note="Description of Artificial Sequence: Synthetic probe"
caaaagatttgtacacagggacattgctgctcg

SEQ ID NO: 258 - DNA, 27 bp, Artificial Sequence
  source: /note="Description of Artificial Sequence: Synthetic probe"
taacggacaagggctgcaatcccacac

SEQ ID NO: 259 - DNA, 33 bp, Artificial Sequence
  source: /note="Description of Artificial Sequence: Synthetic probe"
tgacccaagtatggaagagaatggtgttgaacg

SEQ ID NO: 260 - DNA, 23 bp, Artificial Sequence
  source: /note="Description of Artificial Sequence: Synthetic probe"
agaggcccaaggcacaagtccag

SEQ ID NO: 261 - DNA, 29 bp, Artificial Sequence
  source: /note="Description of Artificial Sequence: Synthetic probe"
acatgcttcaggagactctgtggtttccc

SEQ ID NO: 262 - DNA, 29 bp, Artificial Sequence
  source: /note="Description of Artificial Sequence: Synthetic probe"
agccatcaatcaggaaagccgggttagta

SEQ ID NO: 263 - DNA, 37 bp, Artificial Sequence
  source: /note="Description of Artificial Sequence: Synthetic probe"
gcttctctaaactccaagccatcttctctacgaagag

SEQ ID NO: 264 - DNA, 37 bp, Artificial Sequence
  source: /note="Description of Artificial Sequence: Synthetic probe"
gtgggatgtctcttcagtttatgacacaatagcttcc

SEQ ID NO: 265 - DNA, 38 bp, Artificial Sequence
  source: /note="Description of Artificial Sequence: Synthetic probe"
actattagagtctttaacacctctgtgtgaagatgaca

SEQ ID NO: 266 - DNA, 36 bp, Artificial Sequence
  source: /note="Description of Artificial Sequence: Synthetic probe"
aggagagaaaccttaccattgtgagaagtgtaacct

SEQ ID NO: 267 - DNA, 36 bp, Artificial Sequence
  source: /note="Description of Artificial Sequence: Synthetic probe"
ggaagtttattaaggccagtgaagcagagatggttt

SEQ ID NO: 268 - DNA, 32 bp, Artificial Sequence
  source: /note="Description of Artificial Sequence: Synthetic probe"
aataacatcgttaacaggtccatgacgggctc

SEQ ID NO: 269 - DNA, 28 bp, Artificial Sequence
  source: /note="Description of Artificial Sequence: Synthetic probe"
acagatcgactccaggtggccatcaaag

SEQ ID NO: 270 - DNA, 25 bp, Artificial Sequence
  source: /note="Description of Artificial Sequence: Synthetic probe"
gctggtcccccttgtcagactcagt

SEQ ID NO: 271 - DNA, 32 bp, Artificial Sequence
  source: /note="Description of Artificial Sequence: Synthetic probe"
ctacactgactttgatgggacaagggtgtaca

SEQ ID NO: 272 - DNA, 23 bp, Artificial Sequence
  source: /note="Description of Artificial Sequence: Synthetic probe"
tcacatgcccactcgaagtcgca

SEQ ID NO: 273 - DNA, 27 bp, Artificial Sequence
  source: /note="Description of Artificial Sequence: Synthetic probe"
ctgactttgatgggacaagggtgtaca

SEQ ID NO: 274 - DNA, 25 bp, Artificial Sequence
  source: /note="Description of Artificial Sequence: Synthetic probe"
ctggtgccctgcttcatgatgaacc

SEQ ID NO: 275 - DNA, 25 bp, Artificial Sequence
  source: /note="Description of Artificial Sequence: Synthetic probe"
cactgactttgatgggacaagggtg

SEQ ID NO: 276 - DNA, 30 bp, Artificial Sequence
  source: /note="Description of Artificial Sequence: Synthetic probe"
agcagtttaagcagctctacgaactcgacg

SEQ ID NO: 277 - DNA, 24 bp, Artificial Sequence
  source: /note="Description of Artificial Sequence: Synthetic probe"
tgcagaagcgagggacacctgtga

SEQ ID NO: 278 - DNA, 28 bp, Artificial Sequence
  source: /note="Description of Artificial Sequence: Synthetic probe"
ccctgcggacccaatacatgaagtacct

SEQ ID NO: 279 - DNA, 24 bp, Artificial Sequence
  source: /note="Description of Artificial Sequence: Synthetic probe"
caacagccaagcctccgaaagccg

SEQ ID NO: 280 - DNA, 33 bp, Artificial Sequence
  source: /note="Description of Artificial Sequence: Synthetic probe"
cggcatcatgtacacaggagttctgtttgctca

SEQ ID NO: 281 - DNA, 24 bp, Artificial Sequence
  source: /note="Description of Artificial Sequence: Synthetic probe"
agtttgccatgtacccaccgtcga

SEQ ID NO: 282 - DNA, 28 bp, Artificial Sequence
  source: /note="Description of Artificial Sequence: Synthetic probe"
ctttaagtttgccatgtacccaccgtcg

SEQ ID NO: 283 - DNA, 25 bp, Artificial Sequence
  source: /note="Description of Artificial Sequence: Synthetic probe"
ttgccatgtacccaccgtcgatgat

SEQ ID NO: 284 - DNA, 28 bp, Artificial Sequence
  source: /note="Description of Artificial Sequence: Synthetic probe"
ttctattgcccagtttccccagccagaa

SEQ ID NO: 285 - DNA, 29 bp, Artificial Sequence
  source: /note="Description of Artificial Sequence: Synthetic probe"
ctcttctattgcccagtttccccagccag

SEQ ID NO: 286 - DNA, 29 bp, Artificial Sequence
  source: /note="Description of Artificial Sequence: Synthetic probe"
ctcctcttctattgcccagtttccccagc

SEQ ID NO: 287 - DNA, 30 bp, Artificial Sequence
  source: /note="Description of Artificial Sequence: Synthetic probe"
tccttcttcatgcaagatggccatcacagc

SEQ ID NO: 288 - DNA, 25 bp, Artificial Sequence
  source: /note="Description of Artificial Sequence: Synthetic probe"
aggacccttacagaggcatgccacc

SEQ ID NO: 289 - DNA, 31 bp, Artificial Sequence
  source: /note="Description of Artificial Sequence: Synthetic probe"
tggagcagcaagtccgagaaaggaatctgaa

SEQ ID NO: 290 - DNA, 29 bp, Artificial Sequence
  source: /note="Description of Artificial Sequence: Synthetic probe"
agaaacctgctgaggtattccggaaggac

SEQ ID NO: 291 - DNA, 34 bp, Artificial Sequence
  source: /note="Description of Artificial Sequence: Synthetic probe"
cacagccttctctcaggattatagctgagaaggt

SEQ ID NO: 292 - DNA, 27 bp, Artificial Sequence
  source: /note="Description of Artificial Sequence: Synthetic probe"
cttgcagaaatgggttgtgggccagtt

SEQ ID NO: 293 - DNA, 24 bp, Artificial Sequence
  source: /note="Description of Artificial Sequence: Synthetic probe"
tgtgtgcatcaggcctgctatggc

SEQ ID NO: 294 - DNA, 28 bp, Artificial Sequence
  source: /note="Description of Artificial Sequence: Synthetic probe"
tgtggatcccagaggtcagcattgcttg

SEQ ID NO: 295 - DNA, 27 bp, Artificial Sequence
  source: /note="Description of Artificial Sequence: Synthetic probe"
aggacctggagagggtccgaaatctgt

SEQ ID NO: 296 - DNA, 35 bp, Artificial Sequence
  source: /note="Description of Artificial Sequence: Synthetic probe"
ccaagaaattgatgcagggcttcctttgacaaatg

SEQ ID NO: 297 - DNA, 31 bp, Artificial Sequence
  source: /note="Description of Artificial Sequence: Synthetic probe"
catgcctagtccagcagattcaaccaactct

SEQ ID NO: 298 - DNA, 32 bp, Artificial Sequence
  source: /note="Description of Artificial Sequence: Synthetic probe"
cctggacctaacagacctaattttccaatggg

SEQ ID NO: 299 - DNA, 32 bp, Artificial Sequence
  source: /note="Description of Artificial Sequence: Synthetic probe"
ttgaagaattcaatgccaaagcgccagacaaa

SEQ ID NO: 300 - DNA, 32 bp, Artificial Sequence
  source: /note="Description of Artificial Sequence: Synthetic probe"
cggatgtggtgaaagatgcatatgaaacagcc

SEQ ID NO: 301 - DNA, 34 bp, Artificial Sequence
  source: /note="Description of Artificial Sequence: Synthetic probe"
caattcctggacttcgggagagataatgcatgtg

SEQ ID NO: 302 - DNA, 34 bp, Artificial Sequence
  source: /note="Description of Artificial Sequence: Synthetic probe"
tgcttcccagaagcaaaaggttattgaagagagg

SEQ ID NO: 303 - DNA, 33 bp, Artificial Sequence
  source: /note="Description of Artificial Sequence: Synthetic probe"
taactgttcctgcaaaaggctctgagtttctgg

SEQ ID NO: 304 - DNA, 33 bp, Artificial Sequence
  source: /note="Description of Artificial Sequence: Synthetic probe"
cggcttcataaacaacaaggagaaatgctgcgc

SEQ ID NO: 305 - DNA, 26 bp, Artificial Sequence
  source: /note="Description of Artificial Sequence: Synthetic probe"
cgaagactgaggagagtccagcctct

SEQ ID NO: 306 - DNA, 27 bp, Artificial Sequence
  source: /note="Description of Artificial Sequence: Synthetic probe"
aacgaagactgaggagagtccagcctc

SEQ ID NO: 307 - DNA, 28 bp, Artificial Sequence
  source: /note="Description of Artificial Sequence: Synthetic probe"
aagactgaggagagtccagcctctgatg

SEQ ID NO: 308 - DNA, 28 bp, Artificial Sequence
  source: /note="Description of Artificial Sequence: Synthetic probe"
ccacaaaagatcagtggtaacccttccc

SEQ ID NO: 309 - DNA, 21 bp, Artificial Sequence
  source: /note="Description of Artificial Sequence: Synthetic probe"
tcctatgcaagccgtgcatcc

SEQ ID NO: 310 - DNA, 28 bp, Artificial Sequence
  source: /note="Description of Artificial Sequence: Synthetic probe"
tgtagaagatgttcagcgtgcagggctt

SEQ ID NO: 311 - DNA, 34 bp, Artificial Sequence
  source: /note="Description of Artificial Sequence: Synthetic probe"
catacagtggctatgaaggttgtgctgtgttaca

SEQ ID NO: 312 - DNA, 32 bp, Artificial Sequence
  source: /note="Description of Artificial Sequence: Synthetic probe"
tgcagctcctctaagagtgtcacttatgagcc

SEQ ID NO: 313 - DNA, 30 bp, Artificial Sequence
  source: /note="Description of Artificial Sequence: Synthetic probe"
tgcagctggctcgatagtcgtaaatgaaga

SEQ ID NO: 314 - DNA, 29 bp, Artificial Sequence
  source: /note="Description of Artificial Sequence: Synthetic probe"
ttcatccaccactcaagagggaccttgtg